European Patent Application EP 4 748 861 A1, published May 27, 2026. Title: 一种双特异性抗体、其药物偶联物及其用途. Applicant: 映恩生物制药（苏州）有限公司. Application CN. The sequence listing filed with the application follows.

SEQUENCE LISTING (96 sequences)

SEQ ID NO: 1 - protein, 5 aa, synthetic construct
TYGMH

SEQ ID NO: 2 - protein, 17 aa, synthetic construct
VIWDDGSYKYYGDSVKG

SEQ ID NO: 3 - protein, 16 aa, synthetic construct
DGITMVRGVMKDYFDY

SEQ ID NO: 4 - protein, 11 aa, synthetic construct
RASQDISSALV

SEQ ID NO: 5 - protein, 7 aa, synthetic construct
DASSLES

SEQ ID NO: 6 - protein, 9 aa, synthetic construct
QQFNSYPLT

SEQ ID NO: 7 - protein, 6 aa, synthetic construct
SAYYWN

SEQ ID NO: 8 - protein, 16 aa, synthetic construct
  VARIANT 10: note = X is Y or F
YISYDGRNNXNPSLKN

SEQ ID NO: 9 - protein, 9 aa, synthetic construct
DGDYDYFDY

SEQ ID NO: 10 - protein, 11 aa, synthetic construct
RASQDISNYLN

SEQ ID NO: 11 - protein, 7 aa, synthetic construct
YTSILHS

SEQ ID NO: 12 - protein, 9 aa, synthetic construct
QQGDTLPPT

SEQ ID NO: 13 - protein, 30 aa, synthetic construct
QVQLVESGGGVVQPGRSLRLSCAASGFTFS

SEQ ID NO: 14 - protein, 14 aa, synthetic construct
WVRQAPGKGLEWVA

SEQ ID NO: 15 - protein, 32 aa, synthetic construct
RFTISRDNSKNTLYLQMNSLRAEDTAVYYCAR

SEQ ID NO: 16 - protein, 11 aa, synthetic construct
WGQGTLVTVSS

SEQ ID NO: 17 - protein, 23 aa, synthetic construct
AIQLTQSPSSLSASVGDRVTITC

SEQ ID NO: 18 - protein, 15 aa, synthetic construct
WYQQKPGKAPKLLIY

SEQ ID NO: 19 - protein, 32 aa, synthetic construct
GVPSRFSGSESGTDFTLTISSLQPEDFATYYC

SEQ ID NO: 20 - protein, 10 aa, synthetic construct
FGGGTKVEIK

SEQ ID NO: 21 - protein, 30 aa, synthetic construct
QVQLQESGPGLVKPSETLSLTCTVSGYSIT

SEQ ID NO: 22 - protein, 14 aa, synthetic construct
WIRQPFGKGLEWMG

SEQ ID NO: 23 - protein, 32 aa, synthetic construct
RVTISRDTSKNQFSLKLSSVTAADTAVYYCAR

SEQ ID NO: 24 - protein, 11 aa, synthetic construct
WGQGTTVTVSS

SEQ ID NO: 25 - protein, 23 aa, synthetic construct
DIQMTQSPSSLSASVGDRVTITC

SEQ ID NO: 26 - protein, 32 aa, synthetic construct
GVPSRFSGSGSGTDYTFTISSLQPEDIATYFC

SEQ ID NO: 27 - protein, 10 aa, synthetic construct
FGGGTKLEIK

SEQ ID NO: 28 - protein, 125 aa, synthetic construct [sequence omitted]

SEQ ID NO: 29 - protein, 107 aa, synthetic construct [sequence omitted]

SEQ ID NO: 30 - protein, 118 aa, synthetic construct
QVQLQESGPGLVKPSETLSLTCTVSGYSITSAYYWNWIRQPFGKGLEWMGYISYDGRNNFNPSLKNRVTISRDTSKNQFSLKLSSVTAADTAVYYCARDGDYDYFDYWGQGTTVTVSS

SEQ ID NO: 31 - protein, 107 aa, synthetic construct
DIQMTQSPSSLSASVGDRVTITCRASQDISNYLNWYQQKPGKAPKLLIYYTSILHSGVPSRFSGSGSGTDYTFTISSLQPEDIATYFCQQGDTLPPTFGGGTKLEIK

SEQ ID NO: 32 - protein, 107 aa, synthetic construct [sequence omitted]

SEQ ID NO: 33 - protein, 105 aa, synthetic construct
SSASTKGPSVFPLAPSSKSTSGGTAALGCLVKDYFPEPVTVSWNSGALTSGVHTFPAVLQSSGLYSLSSVVTVPSSSLGTQTYICNVNHKPSNTKVDKKVEPKSC

SEQ ID NO: 34 - protein, 103 aa, synthetic construct
ASTKGPSVFPLAPSSKSTSGGTAALGCLVKDYFPEPVTVSWNSGALTSGVHTFPAVLQSSGLYSLSSVVTVPSSSLGTQTYICNVNHKPSNTKVDKKVEPKSC

SEQ ID NO: 35 - protein, 107 aa, synthetic construct
ASVAAPSVFIFPPSDEQLKSGTASVVCLLNNFYPREAKVQWKVDNALQSGNSQESVTEQDSKDSTYSLSSTLTLSKADYEKHKVYACEVTHQGLSSPVTKSFNRGEC

SEQ ID NO: 36 - protein, 209 aa, synthetic construct
SVFLFPPKPKDTLMISRTPEVTCVVVDVSHEDPEVKFNWYVDGVEVHNAKTKPREEQYNSTYRVVSVLTVLHQDWLNGKEYKCKVSNKALPAPIEKTISKAKGQPREPQVYTLPPSRDELTKNQVSLTCLVKGFYPSDIAVEWESNGQPENNYKTTPPVLDSDGSFFLYSKLTVDKSRWQQGNVFSCSVMHEALHNHYTQKSLSLSPGK

SEQ ID NO: 37 - protein, 455 aa, synthetic construct
QVQLVESGGGVVQPGRSLRLSCAASGFTFSTYGMHWVRQAPGKGLEWVAVIWDDGSYKYYGDSVKGRFTISRDNSKNTLYLQMNSLRAEDTAVYYCARDGITMVRGVMKDYFDYWGQGTLVTVSSASTKGPSVFPLAPSSKSTSGGTAALGCLVKDYFPEPVTVSWNSGALTSGVHTFPAVLQSSGLYSLSSVVTVPSSSLGTQTYICNVNHKPSNTKVDKKVEPKSCDKTHTCPPCPAPELLGGPSVFLFPPKPKDTLMISRTPEVTCVVVDVSHEDPEVKFNWYVDGVEVHNAKTKPREEQYNSTYRVVSVLTVLHQDWLNGKEYKCKVSNKALPAPIEKTISKAKGQPREPQVYTLPPSRDELTKNQVSLWCLVKGFYPSDIAVEWESNGQPENNYKTTPPVLDSDGSFFLYSKLTVDKSRWQQGNVFSCSVMHEALHNHYTQKSLSLSPGK

SEQ ID NO: 38 - protein, 214 aa, synthetic construct
AIQLTQSPSSLSASVGDRVTITCRASQDISSALVWYQQKPGKAPKLLIYDASSLESGVPSRFSGSESGTDFTLTISSLQPEDFATYYCQQFNSYPLTFGGGTKVEIKRTVAAPSVFIFPPSDEQLKSGTASVVCLLNNFYPREAKVQWKVDNALQSGNSQESVTEQDSKDSTYSLSSTLTLSKADYEKHKVYACEVTHQGLSSPVTKSFNRGEC

SEQ ID NO: 39 - protein, 452 aa, synthetic construct
QVQLQESGPGLVKPSETLSLTCTVSGYSITSAYYWNWIRQPFGKGLEWMGYISYDGRNNFNPSLKNRVTISRDTSKNQFSLKLSSVTAADTAVYYCARDGDYDYFDYWGQGTTVTVSSASVAAPSVFIFPPSDEQLKSGTASVVCLLNNFYPREAKVQWKVDNALQSGNSQESVTEQDSKDSTYSLSSTLTLSKADYEKHKVYACEVTHQGLSSPVTKSFNRGECDKTHTCPPCPAPELLGGPSVFLFPPKPKDTLMISRTPEVTCVVVDVSHEDPEVKFNWYVDGVEVHNAKTKPREEQYNSTYRVVSVLTVLHQDWLNGKEYKCKVSNKALPAPIEKTISKAKGQPREPQVYTLPPSRDELTKNQVSLSCAVKGFYPSDIAVEWESNGQPENNYKTTPPVLDSDGSFFLVSKLTVDKSRWQQGNVFSCSVMHEALHNHYTQKSLSLSPGK

SEQ ID NO: 40 - protein, 212 aa, synthetic construct
DIQMTQSPSSLSASVGDRVTITCRASQDISNYLNWYQQKPGKAPKLLIYYTSILHSGVPSRFSGSGSGTDYTFTISSLQPEDIATYFCQQGDTLPPTFGGGTKLEIKSSASTKGPSVFPLAPSSKSTSGGTAALGCLVKDYFPEPVTVSWNSGALTSGVHTFPAVLQSSGLYSLSSVVTVPSSSLGTQTYICNVNHKPSNTKVDKKVEPKSC

SEQ ID NO: 41 - protein, 455 aa, synthetic construct
QVQLVESGGGVVQPGRSLRLSCAASGFTFSTYGMHWVRQAPGKGLEWVAVIWDDGSYKYYGDSVKGRFTISRDNSKNTLYLQMNSLRAEDTAVYYCARDGITMVRGVMKDYFDYWGQGTLVTVSSASTKGPSVFPLAPSSKSTSGGTAALGCLVKDYFPEPVTVSWNSGALTSGVHTFPAVLQSSGLYSLSSVVTVPSSSLGTQTYICNVNHKPSNTKVDKKVEPKSCDKTHTCPPCPAPELLGGPSVFLFPPKPKDTLMISRTPEVTCVVVDVSHEDPEVKFNWYVDGVEVHNAKTKPREEQYNSTYRVVSVLTVLHQDWLNGKEYKCKVSNKALPAPIEKTISKAKGQPREPQVYTLPPCRDELTKNQVSLWCLVKGFYPSDIAVEWESNGQPENNYKTTPPVLDSDGSFFLYSKLTVDKSRWQQGNVFSCSVMHEALHNHYTQKSLSLSPGK

SEQ ID NO: 42 - protein, 452 aa, synthetic construct
QVQLQESGPGLVKPSETLSLTCTVSGYSITSAYYWNWIRQPFGKGLEWMGYISYDGRNNFNPSLKNRVTISRDTSKNQFSLKLSSVTAADTAVYYCARDGDYDYFDYWGQGTTVTVSSASVAAPSVFIFPPSDEQLKSGTASVVCLLNNFYPREAKVQWKVDNALQSGNSQESVTEQDSKDSTYSLSSTLTLSKADYEKHKVYACEVTHQGLSSPVTKSFNRGECDKTHTCPPCPAPELLGGPSVFLFPPKPKDTLMISRTPEVTCVVVDVSHEDPEVKFNWYVDGVEVHNAKTKPREEQYNSTYRVVSVLTVLHQDWLNGKEYKCKVSNKALPAPIEKTISKAKGQPREPQVCTLPPSRDELTKNQVSLSCAVKGFYPSDIAVEWESNGQPENNYKTTPPVLDSDGSFFLVSKLTVDKSRWQQGNVFSCSVMHEALHNHYTQKSLSLSPGK

SEQ ID NO: 43 - protein, 455 aa, synthetic construct
QVQLVESGGGVVQPGRSLRLSCAASGFTFSTYGMHWVRQAPGKGLEWVAVIWDDGSYKYYGDSVKGRFTISRDNSKNTLYLQMNSLRAEDTAVYYCARDGITMVRGVMKDYFDYWGQGTLVTVSSASTKGPSVFPLAPSSKSTSGGTAALGCLVKDYFPEPVTVSWNSGALTSGVHTFPAVLQSSGLYSLSSVVTVPSSSLGTQTYICNVNHKPSNTKVDKKVEPKSCDKTHTCPPCPAPELLGGPSVFLFPPKPKDTLMISRTPEVTCVVVDVSHEDPEVKFNWYVDGVEVHNAKTKPREEQYNSTYRVVSVLTVLHQDWLNGKEYKCKVSNKALPAPIEKTISKAKGQPREPQVYTLPPSRDELTKNQVSLSCAVKGFYPSDIAVEWESNGQPENNYKTTPPVLDSDGSFFLVSKLTVDKSRWQQGNVFSCSVMHEALHNHYTQKSLSLSPGK

SEQ ID NO: 44 - protein, 452 aa, synthetic construct
QVQLQESGPGLVKPSETLSLTCTVSGYSITSAYYWNWIRQPFGKGLEWMGYISYDGRNNFNPSLKNRVTISRDTSKNQFSLKLSSVTAADTAVYYCARDGDYDYFDYWGQGTTVTVSSASVAAPSVFIFPPSDEQLKSGTASVVCLLNNFYPREAKVQWKVDNALQSGNSQESVTEQDSKDSTYSLSSTLTLSKADYEKHKVYACEVTHQGLSSPVTKSFNRGECDKTHTCPPCPAPELLGGPSVFLFPPKPKDTLMISRTPEVTCVVVDVSHEDPEVKFNWYVDGVEVHNAKTKPREEQYNSTYRVVSVLTVLHQDWLNGKEYKCKVSNKALPAPIEKTISKAKGQPREPQVYTLPPSRDELTKNQVSLWCLVKGFYPSDIAVEWESNGQPENNYKTTPPVLDSDGSFFLYSKLTVDKSRWQQGNVFSCSVMHEALHNHYTQKSLSLSPGK

SEQ ID NO: 45 - protein, 455 aa, synthetic construct
QVQLVESGGGVVQPGRSLRLSCAASGFTFSTYGMHWVRQAPGKGLEWVAVIWDDGSYKYYGDSVKGRFTISRDNSKNTLYLQMNSLRAEDTAVYYCARDGITMVRGVMKDYFDYWGQGTLVTVSSASTKGPSVFPLAPSSKSTSGGTAALGCLVKDYFPEPVTVSWNSGALTSGVHTFPAVLQSSGLYSLSSVVTVPSSSLGTQTYICNVNHKPSNTKVDKKVEPKSCDKTHTCPPCPAPELLGGPSVFLFPPKPKDTLMISRTPEVTCVVVDVSHEDPEVKFNWYVDGVEVHNAKTKPREEQYNSTYRVVSVLTVLHQDWLNGKEYKCKVSNKALPAPIEKTISKAKGQPREPQVCTLPPSRDELTKNQVSLSCAVKGFYPSDIAVEWESNGQPENNYKTTPPVLDSDGSFFLVSKLTVDKSRWQQGNVFSCSVMHEALHNHYTQKSLSLSPGK

SEQ ID NO: 46 - protein, 452 aa, synthetic construct
QVQLQESGPGLVKPSETLSLTCTVSGYSITSAYYWNWIRQPFGKGLEWMGYISYDGRNNFNPSLKNRVTISRDTSKNQFSLKLSSVTAADTAVYYCARDGDYDYFDYWGQGTTVTVSSASVAAPSVFIFPPSDEQLKSGTASVVCLLNNFYPREAKVQWKVDNALQSGNSQESVTEQDSKDSTYSLSSTLTLSKADYEKHKVYACEVTHQGLSSPVTKSFNRGECDKTHTCPPCPAPELLGGPSVFLFPPKPKDTLMISRTPEVTCVVVDVSHEDPEVKFNWYVDGVEVHNAKTKPREEQYNSTYRVVSVLTVLHQDWLNGKEYKCKVSNKALPAPIEKTISKAKGQPREPQVYTLPPCRDELTKNQVSLWCLVKGFYPSDIAVEWESNGQPENNYKTTPPVLDSDGSFFLYSKLTVDKSRWQQGNVFSCSVMHEALHNHYTQKSLSLSPGK

SEQ ID NO: 47 - protein, 459 aa, synthetic construct
QVQLVESGGGVVQPGRSLRLSCAASGFTFSTYGMHWVRQAPGKGLEWVAVIWDDGSYKYYGDSVKGRFTISRDNSKNTLYLQMNSLRAEDTAVYYCARDGITMVRGVMKDYFDYWGQGTLVTVSSASVAAPSVFIFPPSDEQLKSGTASVVCLLNNFYPREAKVQWKVDNALQSGNSQESVTEQDSKDSTYSLSSTLTLSKADYEKHKVYACEVTHQGLSSPVTKSFNRGECDKTHTCPPCPAPELLGGPSVFLFPPKPKDTLMISRTPEVTCVVVDVSHEDPEVKFNWYVDGVEVHNAKTKPREEQYNSTYRVVSVLTVLHQDWLNGKEYKCKVSNKALPAPIEKTISKAKGQPREPQVYTLPPSRDELTKNQVSLWCLVKGFYPSDIAVEWESNGQPENNYKTTPPVLDSDGSFFLYSKLTVDKSRWQQGNVFSCSVMHEALHNHYTQKSLSLSPGK

SEQ ID NO: 48 - protein, 212 aa, synthetic construct
AIQLTQSPSSLSASVGDRVTITCRASQDISSALVWYQQKPGKAPKLLIYDASSLESGVPSRFSGSESGTDFTLTISSLQPEDFATYYCQQFNSYPLTFGGGTKVEIKSSASTKGPSVFPLAPSSKSTSGGTAALGCLVKDYFPEPVTVSWNSGALTSGVHTFPAVLQSSGLYSLSSVVTVPSSSLGTQTYICNVNHKPSNTKVDKKVEPKSC

SEQ ID NO: 49 - protein, 448 aa, synthetic construct
QVQLQESGPGLVKPSETLSLTCTVSGYSITSAYYWNWIRQPFGKGLEWMGYISYDGRNNFNPSLKNRVTISRDTSKNQFSLKLSSVTAADTAVYYCARDGDYDYFDYWGQGTTVTVSSASTKGPSVFPLAPSSKSTSGGTAALGCLVKDYFPEPVTVSWNSGALTSGVHTFPAVLQSSGLYSLSSVVTVPSSSLGTQTYICNVNHKPSNTKVDKKVEPKSCDKTHTCPPCPAPELLGGPSVFLFPPKPKDTLMISRTPEVTCVVVDVSHEDPEVKFNWYVDGVEVHNAKTKPREEQYNSTYRVVSVLTVLHQDWLNGKEYKCKVSNKALPAPIEKTISKAKGQPREPQVYTLPPSRDELTKNQVSLSCAVKGFYPSDIAVEWESNGQPENNYKTTPPVLDSDGSFFLVSKLTVDKSRWQQGNVFSCSVMHEALHNHYTQKSLSLSPGK

SEQ ID NO: 50 - protein, 214 aa, synthetic construct
DIQMTQSPSSLSASVGDRVTITCRASQDISNYLNWYQQKPGKAPKLLIYYTSILHSGVPSRFSGSGSGTDYTFTISSLQPEDIATYFCQQGDTLPPTFGGGTKLEIKRTVAAPSVFIFPPSDEQLKSGTASVVCLLNNFYPREAKVQWKVDNALQSGNSQESVTEQDSKDSTYSLSSTLTLSKADYEKHKVYACEVTHQGLSSPVTKSFNRGEC

SEQ ID NO: 51 - protein, 459 aa, synthetic construct
QVQLVESGGGVVQPGRSLRLSCAASGFTFSTYGMHWVRQAPGKGLEWVAVIWDDGSYKYYGDSVKGRFTISRDNSKNTLYLQMNSLRAEDTAVYYCARDGITMVRGVMKDYFDYWGQGTLVTVSSASVAAPSVFIFPPSDEQLKSGTASVVCLLNNFYPREAKVQWKVDNALQSGNSQESVTEQDSKDSTYSLSSTLTLSKADYEKHKVYACEVTHQGLSSPVTKSFNRGECDKTHTCPPCPAPELLGGPSVFLFPPKPKDTLMISRTPEVTCVVVDVSHEDPEVKFNWYVDGVEVHNAKTKPREEQYNSTYRVVSVLTVLHQDWLNGKEYKCKVSNKALPAPIEKTISKAKGQPREPQVYTLPPCRDELTKNQVSLWCLVKGFYPSDIAVEWESNGQPENNYKTTPPVLDSDGSFFLYSKLTVDKSRWQQGNVFSCSVMHEALHNHYTQKSLSLSPGK

SEQ ID NO: 52 - protein, 448 aa, synthetic construct
QVQLQESGPGLVKPSETLSLTCTVSGYSITSAYYWNWIRQPFGKGLEWMGYISYDGRNNFNPSLKNRVTISRDTSKNQFSLKLSSVTAADTAVYYCARDGDYDYFDYWGQGTTVTVSSASTKGPSVFPLAPSSKSTSGGTAALGCLVKDYFPEPVTVSWNSGALTSGVHTFPAVLQSSGLYSLSSVVTVPSSSLGTQTYICNVNHKPSNTKVDKKVEPKSCDKTHTCPPCPAPELLGGPSVFLFPPKPKDTLMISRTPEVTCVVVDVSHEDPEVKFNWYVDGVEVHNAKTKPREEQYNSTYRVVSVLTVLHQDWLNGKEYKCKVSNKALPAPIEKTISKAKGQPREPQVCTLPPSRDELTKNQVSLSCAVKGFYPSDIAVEWESNGQPENNYKTTPPVLDSDGSFFLVSKLTVDKSRWQQGNVFSCSVMHEALHNHYTQKSLSLSPGK

SEQ ID NO: 53 - protein, 459 aa, synthetic construct
QVQLVESGGGVVQPGRSLRLSCAASGFTFSTYGMHWVRQAPGKGLEWVAVIWDDGSYKYYGDSVKGRFTISRDNSKNTLYLQMNSLRAEDTAVYYCARDGITMVRGVMKDYFDYWGQGTLVTVSSASVAAPSVFIFPPSDEQLKSGTASVVCLLNNFYPREAKVQWKVDNALQSGNSQESVTEQDSKDSTYSLSSTLTLSKADYEKHKVYACEVTHQGLSSPVTKSFNRGECDKTHTCPPCPAPELLGGPSVFLFPPKPKDTLMISRTPEVTCVVVDVSHEDPEVKFNWYVDGVEVHNAKTKPREEQYNSTYRVVSVLTVLHQDWLNGKEYKCKVSNKALPAPIEKTISKAKGQPREPQVYTLPPSRDELTKNQVSLSCAVKGFYPSDIAVEWESNGQPENNYKTTPPVLDSDGSFFLVSKLTVDKSRWQQGNVFSCSVMHEALHNHYTQKSLSLSPGK

SEQ ID NO: 54 - protein, 448 aa, synthetic construct
QVQLQESGPGLVKPSETLSLTCTVSGYSITSAYYWNWIRQPFGKGLEWMGYISYDGRNNFNPSLKNRVTISRDTSKNQFSLKLSSVTAADTAVYYCARDGDYDYFDYWGQGTTVTVSSASTKGPSVFPLAPSSKSTSGGTAALGCLVKDYFPEPVTVSWNSGALTSGVHTFPAVLQSSGLYSLSSVVTVPSSSLGTQTYICNVNHKPSNTKVDKKVEPKSCDKTHTCPPCPAPELLGGPSVFLFPPKPKDTLMISRTPEVTCVVVDVSHEDPEVKFNWYVDGVEVHNAKTKPREEQYNSTYRVVSVLTVLHQDWLNGKEYKCKVSNKALPAPIEKTISKAKGQPREPQVYTLPPSRDELTKNQVSLWCLVKGFYPSDIAVEWESNGQPENNYKTTPPVLDSDGSFFLYSKLTVDKSRWQQGNVFSCSVMHEALHNHYTQKSLSLSPGK

SEQ ID NO: 55 - protein, 459 aa, synthetic construct
QVQLVESGGGVVQPGRSLRLSCAASGFTFSTYGMHWVRQAPGKGLEWVAVIWDDGSYKYYGDSVKGRFTISRDNSKNTLYLQMNSLRAEDTAVYYCARDGITMVRGVMKDYFDYWGQGTLVTVSSASVAAPSVFIFPPSDEQLKSGTASVVCLLNNFYPREAKVQWKVDNALQSGNSQESVTEQDSKDSTYSLSSTLTLSKADYEKHKVYACEVTHQGLSSPVTKSFNRGECDKTHTCPPCPAPELLGGPSVFLFPPKPKDTLMISRTPEVTCVVVDVSHEDPEVKFNWYVDGVEVHNAKTKPREEQYNSTYRVVSVLTVLHQDWLNGKEYKCKVSNKALPAPIEKTISKAKGQPREPQVCTLPPSRDELTKNQVSLSCAVKGFYPSDIAVEWESNGQPENNYKTTPPVLDSDGSFFLVSKLTVDKSRWQQGNVFSCSVMHEALHNHYTQKSLSLSPGK

SEQ ID NO: 56 - protein, 448 aa, synthetic construct
QVQLQESGPGLVKPSETLSLTCTVSGYSITSAYYWNWIRQPFGKGLEWMGYISYDGRNNFNPSLKNRVTISRDTSKNQFSLKLSSVTAADTAVYYCARDGDYDYFDYWGQGTTVTVSSASTKGPSVFPLAPSSKSTSGGTAALGCLVKDYFPEPVTVSWNSGALTSGVHTFPAVLQSSGLYSLSSVVTVPSSSLGTQTYICNVNHKPSNTKVDKKVEPKSCDKTHTCPPCPAPELLGGPSVFLFPPKPKDTLMISRTPEVTCVVVDVSHEDPEVKFNWYVDGVEVHNAKTKPREEQYNSTYRVVSVLTVLHQDWLNGKEYKCKVSNKALPAPIEKTISKAKGQPREPQVYTLPPCRDELTKNQVSLWCLVKGFYPSDIAVEWESNGQPENNYKTTPPVLDSDGSFFLYSKLTVDKSRWQQGNVFSCSVMHEALHNHYTQKSLSLSPGK

SEQ ID NO: 57 - protein, 452 aa, synthetic construct
QVQLQESGPGLVKPSDTLSLTCTVSGYSITSAYYWNWIRQPFGKGLEWMGYISYDGRNNFNPSLKNRVTISRDTSKNQFSLKLDSVTAADTAVYYCARDGDYDYFDYWGQGTTVTVSSASVAAPSVFIFPPSDEQLKSGTASVVCLLNNFYPREAKVQWKVDNALQSGNSQESVTEQDSKDSTYSLSSTLTLSKADYEKHKVYACEVTHQGLSSPVTKSFNRGECDKTHTCPPCPAPELLGGPSVFLFPPKPKDTLMISRTPEVTCVVVDVSHEDPEVKFNWYVDGVEVHNAKTKPREEQYNSTYRVVSVLTVLHQDWLNGKEYKCKVSNKALPAPIEKTISKAKGQPREPQVYTLPPSRDELTKNQVSLSCAVKGFYPSDIAVEWESNGQPENNYKTTPPVLDSDGSFFLVSKLTVDKSRWQQGNVFSCSVMHEALHNHYTQKSLSLSPGK

SEQ ID NO: 58 - protein, 212 aa, synthetic construct
DIQMTQSPDSLSASLGDRVTITCRASQDISNYLNWYQQKPGKAPKLLIYYTSILHSGVPSRFSGSGSGTDYTFTISSLQPEDIATYFCQQGDTLPPTFGGGTKLEIKSSASTKGPSVFPLAPSSKSTSGGTAALGCLVKDYFPEPVTVSWNSGALTSGVHTFPAVLQSSGLYSLSSVVTVPSSSLGTQTYICNVNHKPSNTKVDKKVEPKSC

SEQ ID NO: 59 - protein, 452 aa, synthetic construct
QVQLQESGPGLVKPSDTLSLTCTVSGYSITSAYYWNWIRQPFGKGLEWMGYISYDGRNNFNPSLKNRVTISRDTSKNQFSLKLDSVTAADTAVYYCARDGDYDYFDYWGQGTTVTVSSASVAAPSVFIFPPSDEQLKSGTASVVCLLNNFYPREAKVQWKVDNALQSGNSQESVTEQDSKDSTYSLSSTLTLSKADYEKHKVYACEVTHQGLSSPVTKSFNRGECDKTHTCPPCPAPELLGGPSVFLFPPKPKDTLMISRTPEVTCVVVDVSHEDPEVKFNWYVDGVEVHNAKTKPREEQYNSTYRVVSVLTVLHQDWLNGKEYKCKVSNKALPAPIEKTISKAKGQPREPQVCTLPPSRDELTKNQVSLSCAVKGFYPSDIAVEWESNGQPENNYKTTPPVLDSDGSFFLVSKLTVDKSRWQQGNVFSCSVMHEALHNHYTQKSLSLSPGK

SEQ ID NO: 60 - protein, 452 aa, synthetic construct
QVQLQESGPGLVKPSDTLSLTCTVSGYSITSAYYWNWIRQPFGKGLEWMGYISYDGRNNFNPSLKNRVTISRDTSKNQFSLKLDSVTAADTAVYYCARDGDYDYFDYWGQGTTVTVSSASVAAPSVFIFPPSDEQLKSGTASVVCLLNNFYPREAKVQWKVDNALQSGNSQESVTEQDSKDSTYSLSSTLTLSKADYEKHKVYACEVTHQGLSSPVTKSFNRGECDKTHTCPPCPAPELLGGPSVFLFPPKPKDTLMISRTPEVTCVVVDVSHEDPEVKFNWYVDGVEVHNAKTKPREEQYNSTYRVVSVLTVLHQDWLNGKEYKCKVSNKALPAPIEKTISKAKGQPREPQVYTLPPSRDELTKNQVSLWCLVKGFYPSDIAVEWESNGQPENNYKTTPPVLDSDGSFFLYSKLTVDKSRWQQGNVFSCSVMHEALHNHYTQKSLSLSPGK

SEQ ID NO: 61 - protein, 452 aa, synthetic construct
QVQLQESGPGLVKPSDTLSLTCTVSGYSITSAYYWNWIRQPFGKGLEWMGYISYDGRNNFNPSLKNRVTISRDTSKNQFSLKLDSVTAADTAVYYCARDGDYDYFDYWGQGTTVTVSSASVAAPSVFIFPPSDEQLKSGTASVVCLLNNFYPREAKVQWKVDNALQSGNSQESVTEQDSKDSTYSLSSTLTLSKADYEKHKVYACEVTHQGLSSPVTKSFNRGECDKTHTCPPCPAPELLGGPSVFLFPPKPKDTLMISRTPEVTCVVVDVSHEDPEVKFNWYVDGVEVHNAKTKPREEQYNSTYRVVSVLTVLHQDWLNGKEYKCKVSNKALPAPIEKTISKAKGQPREPQVYTLPPCRDELTKNQVSLWCLVKGFYPSDIAVEWESNGQPENNYKTTPPVLDSDGSFFLYSKLTVDKSRWQQGNVFSCSVMHEALHNHYTQKSLSLSPGK

SEQ ID NO: 62 - protein, 448 aa, synthetic construct
QVQLQESGPGLVKPSDTLSLTCTVSGYSITSAYYWNWIRQPFGKGLEWMGYISYDGRNNFNPSLKNRVTISRDTSKNQFSLKLDSVTAADTAVYYCARDGDYDYFDYWGQGTTVTVSSASTKGPSVFPLAPSSKSTSGGTAALGCLVKDYFPEPVTVSWNSGALTSGVHTFPAVLQSSGLYSLSSVVTVPSSSLGTQTYICNVNHKPSNTKVDKKVEPKSCDKTHTCPPCPAPELLGGPSVFLFPPKPKDTLMISRTPEVTCVVVDVSHEDPEVKFNWYVDGVEVHNAKTKPREEQYNSTYRVVSVLTVLHQDWLNGKEYKCKVSNKALPAPIEKTISKAKGQPREPQVYTLPPSRDELTKNQVSLSCAVKGFYPSDIAVEWESNGQPENNYKTTPPVLDSDGSFFLVSKLTVDKSRWQQGNVFSCSVMHEALHNHYTQKSLSLSPGK

SEQ ID NO: 63 - protein, 214 aa, synthetic construct
DIQMTQSPDSLSASLGDRVTITCRASQDISNYLNWYQQKPGKAPKLLIYYTSILHSGVPSRFSGSGSGTDYTFTISSLQPEDIATYFCQQGDTLPPTFGGGTKLEIKRTVAAPSVFIFPPSDEQLKSGTASVVCLLNNFYPREAKVQWKVDNALQSGNSQESVTEQDSKDSTYSLSSTLTLSKADYEKHKVYACEVTHQGLSSPVTKSFNRGEC

SEQ ID NO: 64 - protein, 448 aa, synthetic construct
QVQLQESGPGLVKPSDTLSLTCTVSGYSITSAYYWNWIRQPFGKGLEWMGYISYDGRNNFNPSLKNRVTISRDTSKNQFSLKLDSVTAADTAVYYCARDGDYDYFDYWGQGTTVTVSSASTKGPSVFPLAPSSKSTSGGTAALGCLVKDYFPEPVTVSWNSGALTSGVHTFPAVLQSSGLYSLSSVVTVPSSSLGTQTYICNVNHKPSNTKVDKKVEPKSCDKTHTCPPCPAPELLGGPSVFLFPPKPKDTLMISRTPEVTCVVVDVSHEDPEVKFNWYVDGVEVHNAKTKPREEQYNSTYRVVSVLTVLHQDWLNGKEYKCKVSNKALPAPIEKTISKAKGQPREPQVCTLPPSRDELTKNQVSLSCAVKGFYPSDIAVEWESNGQPENNYKTTPPVLDSDGSFFLVSKLTVDKSRWQQGNVFSCSVMHEALHNHYTQKSLSLSPGK

SEQ ID NO: 65 - protein, 448 aa, synthetic construct
QVQLQESGPGLVKPSDTLSLTCTVSGYSITSAYYWNWIRQPFGKGLEWMGYISYDGRNNFNPSLKNRVTISRDTSKNQFSLKLDSVTAADTAVYYCARDGDYDYFDYWGQGTTVTVSSASTKGPSVFPLAPSSKSTSGGTAALGCLVKDYFPEPVTVSWNSGALTSGVHTFPAVLQSSGLYSLSSVVTVPSSSLGTQTYICNVNHKPSNTKVDKKVEPKSCDKTHTCPPCPAPELLGGPSVFLFPPKPKDTLMISRTPEVTCVVVDVSHEDPEVKFNWYVDGVEVHNAKTKPREEQYNSTYRVVSVLTVLHQDWLNGKEYKCKVSNKALPAPIEKTISKAKGQPREPQVYTLPPSRDELTKNQVSLWCLVKGFYPSDIAVEWESNGQPENNYKTTPPVLDSDGSFFLYSKLTVDKSRWQQGNVFSCSVMHEALHNHYTQKSLSLSPGK

SEQ ID NO: 66 - protein, 448 aa, synthetic construct
QVQLQESGPGLVKPSDTLSLTCTVSGYSITSAYYWNWIRQPFGKGLEWMGYISYDGRNNFNPSLKNRVTISRDTSKNQFSLKLDSVTAADTAVYYCARDGDYDYFDYWGQGTTVTVSSASTKGPSVFPLAPSSKSTSGGTAALGCLVKDYFPEPVTVSWNSGALTSGVHTFPAVLQSSGLYSLSSVVTVPSSSLGTQTYICNVNHKPSNTKVDKKVEPKSCDKTHTCPPCPAPELLGGPSVFLFPPKPKDTLMISRTPEVTCVVVDVSHEDPEVKFNWYVDGVEVHNAKTKPREEQYNSTYRVVSVLTVLHQDWLNGKEYKCKVSNKALPAPIEKTISKAKGQPREPQVYTLPPCRDELTKNQVSLWCLVKGFYPSDIAVEWESNGQPENNYKTTPPVLDSDGSFFLYSKLTVDKSRWQQGNVFSCSVMHEALHNHYTQKSLSLSPGK

SEQ ID NO: 67 - protein, 452 aa, synthetic construct
QVQLQESGPGLVKPSDTLSLTCTVSGYSITSAYYWNWIRQPFGKGLEWMGYISYDGRNNYNPSLKNRVTISRDTSKNQFSLKLDSVTAADTAVYYCARDGDYDYFDYWGQGTTVTVSSASVAAPSVFIFPPSDEQLKSGTASVVCLLNNFYPREAKVQWKVDNALQSGNSQESVTEQDSKDSTYSLSSTLTLSKADYEKHKVYACEVTHQGLSSPVTKSFNRGECDKTHTCPPCPAPELLGGPSVFLFPPKPKDTLMISRTPEVTCVVVDVSHEDPEVKFNWYVDGVEVHNAKTKPREEQYNSTYRVVSVLTVLHQDWLNGKEYKCKVSNKALPAPIEKTISKAKGQPREPQVYTLPPSRDELTKNQVSLSCAVKGFYPSDIAVEWESNGQPENNYKTTPPVLDSDGSFFLVSKLTVDKSRWQQGNVFSCSVMHEALHNHYTQKSLSLSPGK

SEQ ID NO: 68 - protein, 212 aa, synthetic construct
DIQMTQEPSSLSASVGDRVTITCRASQDISNYLNWYQQKPGKAPKLLIYYTSILHSGVPSRFSGSGSGTDYTFTISSLQPEDIATYFCQQGDTLPPTFGGGTKLEIKSSASTKGPSVFPLAPSSKSTSGGTAALGCLVKDYFPEPVTVSWNSGALTSGVHTFPAVLQSSGLYSLSSVVTVPSSSLGTQTYICNVNHKPSNTKVDKKVEPKSC

SEQ ID NO: 69 - protein, 452 aa, synthetic construct
QVQLQESGPGLVKPSDTLSLTCTVSGYSITSAYYWNWIRQPFGKGLEWMGYISYDGRNNYNPSLKNRVTISRDTSKNQFSLKLDSVTAADTAVYYCARDGDYDYFDYWGQGTTVTVSSASVAAPSVFIFPPSDEQLKSGTASVVCLLNNFYPREAKVQWKVDNALQSGNSQESVTEQDSKDSTYSLSSTLTLSKADYEKHKVYACEVTHQGLSSPVTKSFNRGECDKTHTCPPCPAPELLGGPSVFLFPPKPKDTLMISRTPEVTCVVVDVSHEDPEVKFNWYVDGVEVHNAKTKPREEQYNSTYRVVSVLTVLHQDWLNGKEYKCKVSNKALPAPIEKTISKAKGQPREPQVCTLPPSRDELTKNQVSLSCAVKGFYPSDIAVEWESNGQPENNYKTTPPVLDSDGSFFLVSKLTVDKSRWQQGNVFSCSVMHEALHNHYTQKSLSLSPGK

SEQ ID NO: 70 - protein, 452 aa, synthetic construct
QVQLQESGPGLVKPSDTLSLTCTVSGYSITSAYYWNWIRQPFGKGLEWMGYISYDGRNNYNPSLKNRVTISRDTSKNQFSLKLDSVTAADTAVYYCARDGDYDYFDYWGQGTTVTVSSASVAAPSVFIFPPSDEQLKSGTASVVCLLNNFYPREAKVQWKVDNALQSGNSQESVTEQDSKDSTYSLSSTLTLSKADYEKHKVYACEVTHQGLSSPVTKSFNRGECDKTHTCPPCPAPELLGGPSVFLFPPKPKDTLMISRTPEVTCVVVDVSHEDPEVKFNWYVDGVEVHNAKTKPREEQYNSTYRVVSVLTVLHQDWLNGKEYKCKVSNKALPAPIEKTISKAKGQPREPQVYTLPPSRDELTKNQVSLWCLVKGFYPSDIAVEWESNGQPENNYKTTPPVLDSDGSFFLYSKLTVDKSRWQQGNVFSCSVMHEALHNHYTQKSLSLSPGK

SEQ ID NO: 71 - protein, 452 aa, synthetic construct
QVQLQESGPGLVKPSDTLSLTCTVSGYSITSAYYWNWIRQPFGKGLEWMGYISYDGRNNYNPSLKNRVTISRDTSKNQFSLKLDSVTAADTAVYYCARDGDYDYFDYWGQGTTVTVSSASVAAPSVFIFPPSDEQLKSGTASVVCLLNNFYPREAKVQWKVDNALQSGNSQESVTEQDSKDSTYSLSSTLTLSKADYEKHKVYACEVTHQGLSSPVTKSFNRGECDKTHTCPPCPAPELLGGPSVFLFPPKPKDTLMISRTPEVTCVVVDVSHEDPEVKFNWYVDGVEVHNAKTKPREEQYNSTYRVVSVLTVLHQDWLNGKEYKCKVSNKALPAPIEKTISKAKGQPREPQVYTLPPCRDELTKNQVSLWCLVKGFYPSDIAVEWESNGQPENNYKTTPPVLDSDGSFFLYSKLTVDKSRWQQGNVFSCSVMHEALHNHYTQKSLSLSPGK

SEQ ID NO: 72 - protein, 448 aa, synthetic construct
QVQLQESGPGLVKPSDTLSLTCTVSGYSITSAYYWNWIRQPFGKGLEWMGYISYDGRNNYNPSLKNRVTISRDTSKNQFSLKLDSVTAADTAVYYCARDGDYDYFDYWGQGTTVTVSSASTKGPSVFPLAPSSKSTSGGTAALGCLVKDYFPEPVTVSWNSGALTSGVHTFPAVLQSSGLYSLSSVVTVPSSSLGTQTYICNVNHKPSNTKVDKKVEPKSCDKTHTCPPCPAPELLGGPSVFLFPPKPKDTLMISRTPEVTCVVVDVSHEDPEVKFNWYVDGVEVHNAKTKPREEQYNSTYRVVSVLTVLHQDWLNGKEYKCKVSNKALPAPIEKTISKAKGQPREPQVYTLPPSRDELTKNQVSLSCAVKGFYPSDIAVEWESNGQPENNYKTTPPVLDSDGSFFLVSKLTVDKSRWQQGNVFSCSVMHEALHNHYTQKSLSLSPGK

SEQ ID NO: 73 - protein, 214 aa, synthetic construct
DIQMTQEPSSLSASVGDRVTITCRASQDISNYLNWYQQKPGKAPKLLIYYTSILHSGVPSRFSGSGSGTDYTFTISSLQPEDIATYFCQQGDTLPPTFGGGTKLEIKRTVAAPSVFIFPPSDEQLKSGTASVVCLLNNFYPREAKVQWKVDNALQSGNSQESVTEQDSKDSTYSLSSTLTLSKADYEKHKVYACEVTHQGLSSPVTKSFNRGEC

SEQ ID NO: 74 - protein, 448 aa, synthetic construct
QVQLQESGPGLVKPSDTLSLTCTVSGYSITSAYYWNWIRQPFGKGLEWMGYISYDGRNNYNPSLKNRVTISRDTSKNQFSLKLDSVTAADTAVYYCARDGDYDYFDYWGQGTTVTVSSASTKGPSVFPLAPSSKSTSGGTAALGCLVKDYFPEPVTVSWNSGALTSGVHTFPAVLQSSGLYSLSSVVTVPSSSLGTQTYICNVNHKPSNTKVDKKVEPKSCDKTHTCPPCPAPELLGGPSVFLFPPKPKDTLMISRTPEVTCVVVDVSHEDPEVKFNWYVDGVEVHNAKTKPREEQYNSTYRVVSVLTVLHQDWLNGKEYKCKVSNKALPAPIEKTISKAKGQPREPQVCTLPPSRDELTKNQVSLSCAVKGFYPSDIAVEWESNGQPENNYKTTPPVLDSDGSFFLVSKLTVDKSRWQQGNVFSCSVMHEALHNHYTQKSLSLSPGK

SEQ ID NO: 75 - protein, 448 aa, synthetic construct
QVQLQESGPGLVKPSDTLSLTCTVSGYSITSAYYWNWIRQPFGKGLEWMGYISYDGRNNYNPSLKNRVTISRDTSKNQFSLKLDSVTAADTAVYYCARDGDYDYFDYWGQGTTVTVSSASTKGPSVFPLAPSSKSTSGGTAALGCLVKDYFPEPVTVSWNSGALTSGVHTFPAVLQSSGLYSLSSVVTVPSSSLGTQTYICNVNHKPSNTKVDKKVEPKSCDKTHTCPPCPAPELLGGPSVFLFPPKPKDTLMISRTPEVTCVVVDVSHEDPEVKFNWYVDGVEVHNAKTKPREEQYNSTYRVVSVLTVLHQDWLNGKEYKCKVSNKALPAPIEKTISKAKGQPREPQVYTLPPSRDELTKNQVSLWCLVKGFYPSDIAVEWESNGQPENNYKTTPPVLDSDGSFFLYSKLTVDKSRWQQGNVFSCSVMHEALHNHYTQKSLSLSPGK

SEQ ID NO: 76 - protein, 448 aa, synthetic construct
QVQLQESGPGLVKPSDTLSLTCTVSGYSITSAYYWNWIRQPFGKGLEWMGYISYDGRNNYNPSLKNRVTISRDTSKNQFSLKLDSVTAADTAVYYCARDGDYDYFDYWGQGTTVTVSSASTKGPSVFPLAPSSKSTSGGTAALGCLVKDYFPEPVTVSWNSGALTSGVHTFPAVLQSSGLYSLSSVVTVPSSSLGTQTYICNVNHKPSNTKVDKKVEPKSCDKTHTCPPCPAPELLGGPSVFLFPPKPKDTLMISRTPEVTCVVVDVSHEDPEVKFNWYVDGVEVHNAKTKPREEQYNSTYRVVSVLTVLHQDWLNGKEYKCKVSNKALPAPIEKTISKAKGQPREPQVYTLPPCRDELTKNQVSLWCLVKGFYPSDIAVEWESNGQPENNYKTTPPVLDSDGSFFLYSKLTVDKSRWQQGNVFSCSVMHEALHNHYTQKSLSLSPGK

SEQ ID NO: 77 - protein, 16 aa, synthetic construct
YISYDGRNNYNPSLKN

SEQ ID NO: 78 - protein, 16 aa, synthetic construct
YISYDGRNNFNPSLKN

SEQ ID NO: 79 - protein, 118 aa, synthetic construct
QVQLQESGPGLVKPSDTLSLTCTVSGYSITSAYYWNWIRQPFGKGLEWMGYISYDGRNNFNPSLKNRVTISRDTSKNQFSLKLDSVTAADTAVYYCARDGDYDYFDYWGQGTTVTVSS

SEQ ID NO: 80 - protein, 118 aa, synthetic construct
QVQLQESGPGLVKPSDTLSLTCTVSGYSITSAYYWNWIRQPFGKGLEWMGYISYDGRNNYNPSLKNRVTISRDTSKNQFSLKLDSVTAADTAVYYCARDGDYDYFDYWGQGTTVTVSS

SEQ ID NO: 81 - protein, 107 aa, synthetic construct
DIQMTQSPDSLSASLGDRVTITCRASQDISNYLNWYQQKPGKAPKLLIYYTSILHSGVPSRFSGSGSGTDYTFTISSLQPEDIATYFCQQGDTLPPTFGGGTKLEIK

SEQ ID NO: 82 - protein, 107 aa, synthetic construct
DIQMTQEPSSLSASVGDRVTITCRASQDISNYLNWYQQKPGKAPKLLIYYTSILHSGVPSRFSGSGSGTDYTFTISSLQPEDIATYFCQQGDTLPPTFGGGTKLEIK

SEQ ID NO: 83 - protein, 455 aa, synthetic construct
QVQLVESGGGVVQPGRSLRLSCAASGFTFSTYGMHWVRQAPGKGLEWVAVIWDDGSYKYYGDSVKGRFTISRDNSKNTLYLQMNSLRAEDTAVYYCARDGITMVRGVMKDYFDYWGQGTLVTVSSASTKGPSVFPLAPSSKSTSGGTAALGCLVKDYFPEPVTVSWNSGALTSGVHTFPAVLQSSGLYSLSSVVTVPSSSLGTQTYICNVNHKPSNTKVDKRVEPKSCDKTHTCPPCPAPELLGGPSVFLFPPKPKDTLMISRTPEVTCVVVDVSHEDPEVKFNWYVDGVEVHNAKTKPREEQYNSTYRVVSVLTVLHQDWLNGKEYKCKVSNKALPAPIEKTISKAKGQPREPQVYTLPPSREEMTKNQVSLTCLVKGFYPSDIAVEWESNGQPENNYKTTPPVLDSDGSFFLYSKLTVDKSRWQQGNVFSCSVMHEALHNHYTQKSLSLSPGK

SEQ ID NO: 84 - protein, 214 aa, synthetic construct; identical to SEQ ID NO: 38

SEQ ID NO: 85 - protein, 448 aa, synthetic construct
QVQLQESGPGLVKPSETLSLTCTVSGYSITSAYYWNWIRQPFGKGLEWMGYISYDGRNNFNPSLKNRVTISRDTSKNQFSLKLSSVTAADTAVYYCARDGDYDYFDYWGQGTTVTVSSASTKGPSVFPLAPSSKSTSGGTAALGCLVKDYFPEPVTVSWNSGALTSGVHTFPAVLQSSGLYSLSSVVTVPSSSLGTQTYICNVNHKPSNTKVDKKVEPKSCDKTHTCPPCPAPELLGGPSVFLFPPKPKDTLMISRTPEVTCVVVDVSHEDPEVKFNWYVDGVEVHNAKTKPREEQYNSTYRVVSVLTVLHQDWLNGKEYKCKVSNKALPAPIEKTISKAKGQPREPQVYTLPPSRDELTKNQVSLTCLVKGFYPSDIAVEWESNGQPENNYKTTPPVLDSDGSFFLYSKLTVDKSRWQQGNVFSCSVMHEALHNHYTQKSLSLSPGK

SEQ ID NO: 86 - protein, 214 aa, synthetic construct; identical to SEQ ID NO: 50

SEQ ID NO: 87 - protein, 449 aa, synthetic construct
QVQLKQSGPGLVQPSQSLSITCTVSGFSLTNYGVHWVRQSPGKGLEWLGVIWSGGNTDYNTPFTSRLSINKDNSKSQVFFKMNSLQSNDTAIYYCARALTYYDYEFAYWGQGTLVTVSAASTKGPSVFPLAPSSKSTSGGTAALGCLVKDYFPEPVTVSWNSGALTSGVHTFPAVLQSSGLYSLSSVVTVPSSSLGTQTYICNVNHKPSNTKVDKKVEPKSCDKTHTCPPCPAPELLGGPSVFLFPPKPKDTLMISRTPEVTCVVVDVSHEDPEVKFNWYVDGVEVHNAKTKPREEQYNSTYRVVSVLTVLHQDWLNGKEYKCKVSNKALPAPIEKTISKAKGQPREPQVYTLPPSRDELTKNQVSLTCLVKGFYPSDIAVEWESNGQPENNYKTTPPVLDSDGSFFLYSKLTVDKSRWQQGNVFSCSVMHEALHNHYTQKSLSLSPGK

SEQ ID NO: 88 - protein, 214 aa, synthetic construct
DILLTQSPVILSVSPGERVSFSCRASQSIGTNIHWYQQRTNGSPRLLIKYASESISGIPSRFSGSGSGTDFTLSINSVESEDIADYYCQQNNNWPTTFGAGTKLELKRTVAAPSVFIFPPSDEQLKSGTASVVCLLNNFYPREAKVQWKVDNALQSGNSQESVTEQDSKDSTYSLSSTLTLSKADYEKHKVYACEVTHQGLSSPVTKSFNRGEC

SEQ ID NO: 89 - protein, 18 aa, synthetic construct
DKTHTCPPCPAPELLGGP

SEQ ID NO: 90 - protein, 477 aa, synthetic construct
DIQMTQSPSSLSASVGDRVTITCRASQDISNYLNWYQQKPGKAPKLLIYYTSILHSGVPSRFSGSGSGTDYTFTISSLQPEDIATYFCQQGDTLPPTFGGGTKLEIKGGGGSGGGGSGGGGSGGGGSQVQLQESGPGLVKPSETLSLTCTVSGYSITSAYYWNWIRQPFGKGLEWMGYISYDGRNNFNPSLKNRVTISRDTSKNQFSLKLSSVTAADTAVYYCARDGDYDYFDYWGQGTTVTVSSEPKSSDKTHTCPPCPAPELLGGPSVFLFPPKPKDTLMISRTPEVTCVVVDVSHEDPEVKFNWYVDGVEVHNAKTKPREEQYNSTYRVVSVLTVLHQDWLNGKEYKCKVSNKALPAPIEKTISKAKGQPREPQVYTLPPSRDELTKNQVSLSCAVKGFYPSDIAVEWESNGQPENNYKTTPPVLDSDGSFFLVSKLTVDKSRWQQGNVFSCSVMHEALHNHYTQKSLSLSPGK

SEQ ID NO: 91 - protein, 702 aa, synthetic construct
QVQLKQSGPGLVQPSQSLSITCTVSGFSLTNYGVHWVRQSPGKGLEWLGVIWSGGNTDYNTPFTSRLSINKDNSKSQVFFKMNSLQSNDTAIYYCARALTYYDYEFAYWGQGTLVTVSSASTKGPSVFPLAPSSKSTSGGTAALGCLVKDYFPEPVTVSWNSGALTSGVHTFPAVLQSSGLYSLSSVVTVPSSSLGTQTYICNVNHKPSNTKVDKRVEPKSCDKTHTCPPCPAPELLGGPSVFLFPPKPKDTLMISRTPEVTCVVVDVSHEDPEVKFNWYVDGVEVHNAKTKPREEQYNSTYRVVSVLTVLHQDWLNGKEYKCKVSNKALPAPIEKTISKAKGQPREPQVYTLPPSRDELTKNQVSLTCLVKGFYPSDIAVEWESNGQPENNYKTTPPVLDSDGSFFLYSKLTVDKSRWQQGNVFSCSVMHEALHNHYTQKSLSLSPGGGGGSGGGGSQVQLQESGGGLVKPGGSLRLSCAASGFTFSSYWMSWVRQAPGKGLEWVANINRDGSASYYVDSVKGRFTISRDDAKNSLYLQMNSLRAEDTAVYYCARDRGVGYFDLWGRGTLVTVSSGGGGSGGGGSGGGGSQSALTQPASVSGSPGQSITISCTGTSSDVGGYNFVSWYQQHPGKAPKLMIYDVSDRPSGVSDRFSGSKSGNTASLIISGLQADDEADYYCSSYGSSSTHVIFGGGTKVTVL

SEQ ID NO: 92 - protein, 214 aa, synthetic construct; identical to SEQ ID NO: 88

SEQ ID NO: 93 - protein, 209 aa, synthetic construct
SVFLFPPKPKDTLMISRTPEVTCVVVDVSHEDPEVKFNWYVDGVEVHNAKTKPREEQYNSTYRVVSVLTVLHQDWLNGKEYKCKVSNKALPAPIEKTISKAKGQPREPQVYTLPPSRDELTKNQVSLWCLVKGFYPSDIAVEWESNGQPENNYKTTPPVLDSDGSFFLYSKLTVDKSRWQQGNVFSCSVMHEALHNHYTQKSLSLSPGK

SEQ ID NO: 94 - protein, 209 aa, synthetic construct
SVFLFPPKPKDTLMISRTPEVTCVVVDVSHEDPEVKFNWYVDGVEVHNAKTKPREEQYNSTYRVVSVLTVLHQDWLNGKEYKCKVSNKALPAPIEKTISKAKGQPREPQVYTLPPSRDELTKNQVSLSCAVKGFYPSDIAVEWESNGQPENNYKTTPPVLDSDGSFFLVSKLTVDKSRWQQGNVFSCSVMHEALHNHYTQKSLSLSPGK

SEQ ID NO: 95 - protein, 20 aa, synthetic construct
GGGGSGGGGSGGGGSGGGGS

SEQ ID NO: 96 - protein, 23 aa, synthetic construct
EPKSSDKTHTCPPCPAPELLGGP